European Patent Specification EP 3 790 946 B1, published October 9, 2024. Title: PROCESS FOR ENZYMATIC OIL DEGUMMING. Applicant: DSM IP Assets B.V. The sequence listing filed with the application follows.

SEQUENCE LISTING (4 sequences)

SEQ ID NO: 1 - protein, 298 aa, Aspergillus niger
  Amino acid sequence of phospholipase A1
MFLRREFGAVAALSVLAHAAPAPAPMQRRDISSTVLDNIDLFAQYSAAAYCSSNIESTGTTLTCDVGNCPLVEAAGATTIDEFDDSSSYGDPTGFIAVDPTNELIVLSFRGSSDLSNWIADLDFGLTSVSSICDGCEMHKGFYEAWEVIADTITSKVEAAVSSYPDYTLVFTGHSYGAALAAVAATVLRNAGYTLDLYNFGQPRIGNLALADYITDQNMGSNYRVTHTDDIVPKLPPELLGYHHFSPEYWITSGNDVTVTTSDVTEVVGVDSTAGNDGTLLDSTTAHRWYTIYISECS

SEQ ID NO: 2 - DNA, 897 bp, Aspergillus niger
  DNA sequence of phospholipase A1 (Genbank: XM_001393495)
atgtttctccgcagggaatttggggctgttgcagccctatctgtgctggcccatgctgctcccgcacctgctccgatgcagcgtagagacatctcctctaccgtcttggacaatatcgacctcttcgcccaatacagtgcagcagcttactgctcctccaacatcgagtccaccggcacgactctgacctgcgacgtaggcaattgccctctcgtcgaggcagccggtgccacgaccatcgatgagtttgacgacagcagcagctacggcgacccgacggggttcatcgccgttgacccgacgaacgagttaatcgttctgtctttccggggcagttccgacctctcgaactggattgccgacctagacttcggcctcacatccgtaagcagcatctgtgatggctgtgagatgcacaagggcttctacgaggcctgggaagtcattgccgacaccatcacatccaaggtggaggccgccgtctccagctatccggactacaccctcgtgttcaccggacacagctacggcgctgcattggcggctgtcgcggccaccgtgctccgcaacgccggatacactcttgacctgtacaacttcggccagccccgtattggcaacctcgccttagccgactacatcaccgaccaaaacatgggcagcaactaccgcgtcacgcacaccgatgacatcgtgcctaagctgcctccggagctgctgggctaccaccacttcagtccggagtactggatcaccagcggcaatgatgtgacggtgacaacgtcggacgtcaccgaggtcgtgggggtggattcgacggctgggaatgacggcacgctgcttgacagtacgactgcccatcggtggtacacgatctacattagtgaatgctcgtag

SEQ ID NO: 3 - protein, 245 aa, Artificial Sequence
  Phospholipase C from WO2005/086900
WSAEDKHNEGINSHLWIVNRAIDIMSRNTTIVNPNETALLNEWRADLENGIYSADYENPYYDDSTYASHFYDPDTGTTYIPFAKHAKETGAKYFNLAGQAYQNQDMQQAFFYLGLSLHYLGDVNQPMHAASFTDLSYPMGFHSKYENFVDTIKNNYIVSDSNGYWNWKGANPEDWIEGAAVAAKQDYPGVVNDTTKDWFVKAAVSQEYADKWRAEVTPVTGKRLMEAQRVTAGYIHLWFDTYVNR

SEQ ID NO: 4 - protein, 298 aa, Artificial Sequence
  Phosphatidylinositol phospholipase C from WO2011/046812
MASSINVLENWSRWMKPINDDIPLARISIPGTHDSGTFKLQNPIKQVWGMTQEYDFRYQMDHGARIFDIRGRLTDDNTIVLHHGPLYLYVTLHEFINEAKQFLKDNPSETIIMSLKKEYEDMKGAESSFSSTFEKNYFRDPIFLKTEGNIKLGDARGKIVLLKRYSGSNESGGYNFFYWPDNETFTSTINGNVNVTVQDKYKVSLDEKINAIKDTLNETINNSEDVNHLYINFTSLSSGGTAWTSPYYYASRINPEIANYIKQKNPTRVGWIIQDFINEKWHPLLYQEVINANKSLVK